European Patent Specification EP 3 455 249 B1, published May 3, 2023. Title: T-Cell Receptors which Recognise Frameshift Mutants of TGFBRII. Applicant: Oslo universitetssykehus HF. The sequence listing filed with the application follows.

SEQUENCE LISTING (82 sequences)

SEQ ID NO: 1 - protein, 9 aa, Homo sapiens
RLSSCVPVA

SEQ ID NO: 2 - protein, 5 aa, Homo sapiens
DSVNN

SEQ ID NO: 3 - protein, 5 aa, Homo sapiens
IPSGT

SEQ ID NO: 4 - protein, 11 aa, Homo sapiens
CAVNAGNMLTF

SEQ ID NO: 5 - protein, 5 aa, Homo sapiens
MDHEN

SEQ ID NO: 6 - protein, 6 aa, Homo sapiens
SYDVKM

SEQ ID NO: 7 - protein, 13 aa, Homo sapiens
CASSSGVTGELFF

SEQ ID NO: 8 - protein, 127 aa, Homo sapiens
MKRILGALLGLLSAQVCCVRGIQVEQSPPDLILQEGANSTLRCNFSDSVNNLQWFHQNPWGQLINLFYIPSGTKQNGRLSATTVATERYSLLYISSSQTTDSGVYFCAVNAGNMLTFGGGTRLMVKP

SEQ ID NO: 9 - protein, 141 aa, Homo sapiens
HIQNPDPAVYQLRDSKSSDKSVCLFTDFDSQTNVSQSKDSDVYITDKTVLDMRSMDFKSNSAVAWSNKSDFACANAFNNSIIPEDTFFPSPESSCDVKLVEKSFETDTNLNFQNLSVIGFRILLLKVAGFNLLMTLRLWSS

SEQ ID NO: 10 - protein, 141 aa, Artificial Sequence
  Cysteine-modified Radium-1 alpha-chain constant region
HIQNPDPAVYQLRDSKSSDKSVCLFTDFDSQTNVSQSKDSDVYITDKCVLDMRSMDFKSNSAVAWSNKSDFACANAFNNSIIPEDTFFPSPESSCDVKLVEKSFETDTNLNFQNLSVIGFRILLLKVAGFNLLMTLRLWSS

SEQ ID NO: 11 - protein, 268 aa, Homo sapiens
MKRILGALLGLLSAQVCCVRGIQVEQSPPDLILQEGANSTLRCNFSDSVNNLQWFHQNPWGQLINLFYIPSGTKQNGRLSATTVATERYSLLYISSSQTTDSGVYFCAVNAGNMLTFGGGTRLMVKPHIQNPDPAVYQLRDSKSSDKSVCLFTDFDSQTNVSQSKDSDVYITDKTVLDMRSMDFKSNSAVAWSNKSDFACANAFNNSIIPEDTFFPSPESSCDVKLVEKSFETDTNLNFQNLSVIGFRILLLKVAGFNLLMTLRLWSS

SEQ ID NO: 12 - protein, 268 aa, Artificial Sequence
  Cysteine-modified Radium-1 alpha-chain
MKRILGALLGLLSAQVCCVRGIQVEQSPPDLILQEGANSTLRCNFSDSVNNLQWFHQNPWGQLINLFYIPSGTKQNGRLSATTVATERYSLLYISSSQTTDSGVYFCAVNAGNMLTFGGGTRLMVKPHIQNPDPAVYQLRDSKSSDKSVCLFTDFDSQTNVSQSKDSDVYITDKCVLDMRSMDFKSNSAVAWSNKSDFACANAFNNSIIPEDTFFPSPESSCDVKLVEKSFETDTNLNFQNLSVIGFRILLLKVAGFNLLMTLRLWSS

SEQ ID NO: 13 - protein, 131 aa, Homo sapiens
MGIRLLCRVAFCFLAVGLVDVKVTQSSRYLVKRTGEKVFLECVQDMDHENMFWYRQDPGLGLRLIYFSYDVKMKEKGDIPEGYSVSREKKERFSLILESASTNQTSMYLCASSSGVTGELFFGEGSRLTVL

SEQ ID NO: 14 - protein, 179 aa, Homo sapiens
EDLKNVFPPEVAVFEPSEAEISHTQKATLVCLATGFYPDHVELSWWVNGKEVHSGVSTDPQPLKEQPALNDSRYCLSSRLRVSATFWQNPRNHFRCQVQFYGLSENDEWTQDRAKPVTQIVSAEAWGRADCGFTSESYQQGVLSATILYEILLGKATLYAVLVSALVLMAMVKRKDSRG

SEQ ID NO: 15 - protein, 179 aa, Artificial Sequence
  Cysteine-modified Radium-1 beta-chain constant region
EDLKNVFPPEVAVFEPSEAEISHTQKATLVCLATGFYPDHVELSWWVNGKEVHSGVCTDPQPLKEQPALNDSRYCLSSRLRVSATFWQNPRNHFRCQVQFYGLSENDEWTQDRAKPVTQIVSAEAWGRADCGFTSESYQQGVLSATILYEILLGKATLYAVLVSALVLMAMVKRKDSRG

SEQ ID NO: 16 - protein, 310 aa, Homo sapiens
MGIRLLCRVAFCFLAVGLVDVKVTQSSRYLVKRTGEKVFLECVQDMDHENMFWYRQDPGLGLRLIYFSYDVKMKEKGDIPEGYSVSREKKERFSLILESASTNQTSMYLCASSSGVTGELFFGEGSRLTVLEDLKNVFPPEVAVFEPSEAEISHTQKATLVCLATGFYPDHVELSWWVNGKEVHSGVSTDPQPLKEQPALNDSRYCLSSRLRVSATFWQNPRNHFRCQVQFYGLSENDEWTQDRAKPVTQIVSAEAWGRADCGFTSESYQQGVLSATILYEILLGKATLYAVLVSALVLMAMVKRKDSRG

SEQ ID NO: 17 - protein, 310 aa, Artificial Sequence
  Cysteine-modified Radium-1 beta-chain
MGIRLLCRVAFCFLAVGLVDVKVTQSSRYLVKRTGEKVFLECVQDMDHENMFWYRQDPGLGLRLIYFSYDVKMKEKGDIPEGYSVSREKKERFSLILESASTNQTSMYLCASSSGVTGELFFGEGSRLTVLEDLKNVFPPEVAVFEPSEAEISHTQKATLVCLATGFYPDHVELSWWVNGKEVHSGVCTDPQPLKEQPALNDSRYCLSSRLRVSATFWQNPRNHFRCQVQFYGLSENDEWTQDRAKPVTQIVSAEAWGRADCGFTSESYQQGVLSATILYEILLGKATLYAVLVSALVLMAMVKRKDSRG

SEQ ID NO: 18 - protein, 26 aa, picornavirus
RAKRGSGATNFSLLKQAGDVEENPGP

SEQ ID NO: 19 - protein, 20 aa, Artificial Sequence
  Double Myc-tag
EQKLISEEDLEQKLISEEDL

SEQ ID NO: 20 - protein, 147 aa, Artificial Sequence
  Radium-1 alpha-chain variable region with double Myc-tag
MKRILGALLGLLSAQVCCVREQKLISEEDLEQKLISEEDLGIQVEQSPPDLILQEGANSTLRCNFSDSVNNLQWFHQNPWGQLINLFYIPSGTKQNGRLSATTVATERYSLLYISSSQTTDSGVYFCAVNAGNMLTFGGGTRLMVKP

SEQ ID NO: 21 - protein, 288 aa, Artificial Sequence
  Radium-1 alpha-chain with double Myc-tag
MKRILGALLGLLSAQVCCVREQKLISEEDLEQKLISEEDLGIQVEQSPPDLILQEGANSTLRCNFSDSVNNLQWFHQNPWGQLINLFYIPSGTKQNGRLSATTVATERYSLLYISSSQTTDSGVYFCAVNAGNMLTFGGGTRLMVKPHIQNPDPAVYQLRDSKSSDKSVCLFTDFDSQTNVSQSKDSDVYITDKTVLDMRSMDFKSNSAVAWSNKSDFACANAFNNSIIPEDTFFPSPESSCDVKLVEKSFETDTNLNFQNLSVIGFRILLLKVAGFNLLMTLRLWSS

SEQ ID NO: 22 - protein, 288 aa, Artificial Sequence
  Cysteine-modified Radium-1 alpha-chain with double Myc-tag
MKRILGALLGLLSAQVCCVREQKLISEEDLEQKLISEEDLGIQVEQSPPDLILQEGANSTLRCNFSDSVNNLQWFHQNPWGQLINLFYIPSGTKQNGRLSATTVATERYSLLYISSSQTTDSGVYFCAVNAGNMLTFGGGTRLMVKPHIQNPDPAVYQLRDSKSSDKSVCLFTDFDSQTNVSQSKDSDVYITDKCVLDMRSMDFKSNSAVAWSNKSDFACANAFNNSIIPEDTFFPSPESSCDVKLVEKSFETDTNLNFQNLSVIGFRILLLKVAGFNLLMTLRLWSS

SEQ ID NO: 23 - protein, 136 aa, Mus musculus
IQNPEPAVYQLKDPRSQDSTLCLFTDFDSQINVPKTMESGTFITDKTVLDMKAMDSKSNGAIAWSNQTSFTCQDIFKETNATYPSSDVPCDATLTEKSFETDMNLNFQNLSVMGLRILLLKVAGFNLLMTLRLWSS

SEQ ID NO: 24 - protein, 136 aa, Artificial Sequence
  Cysteine-modified murinised Radium-1 alpha chain constant region
IQNPEPAVYQLKDPRSQDSTLCLFTDFDSQINVPKTMESGTFITDKCVLDMKAMDSKSNGAIAWSNQTSFTCQDIFKETNATYPSSDVPCDATLTEKSFETDMNLNFQNLSVMGLRILLLKVAGFNLLMTLRLWSS

SEQ ID NO: 25 - protein, 263 aa, Artificial Sequence
  Radium-1 alpha-chain with murinised constant region
MKRILGALLGLLSAQVCCVRGIQVEQSPPDLILQEGANSTLRCNFSDSVNNLQWFHQNPWGQLINLFYIPSGTKQNGRLSATTVATERYSLLYISSSQTTDSGVYFCAVNAGNMLTFGGGTRLMVKPIQNPEPAVYQLKDPRSQDSTLCLFTDFDSQINVPKTMESGTFITDKTVLDMKAMDSKSNGAIAWSNQTSFTCQDIFKETNATYPSSDVPCDATLTEKSFETDMNLNFQNLSVMGLRILLLKVAGFNLLMTLRLWSS

SEQ ID NO: 26 - protein, 263 aa, Artificial Sequence
  Radium-1 alpha-chain with cysteine-modified murinised constant region
MKRILGALLGLLSAQVCCVRGIQVEQSPPDLILQEGANSTLRCNFSDSVNNLQWFHQNPWGQLINLFYIPSGTKQNGRLSATTVATERYSLLYISSSQTTDSGVYFCAVNAGNMLTFGGGTRLMVKPIQNPEPAVYQLKDPRSQDSTLCLFTDFDSQINVPKTMESGTFITDKCVLDMKAMDSKSNGAIAWSNQTSFTCQDIFKETNATYPSSDVPCDATLTEKSFETDMNLNFQNLSVMGLRILLLKVAGFNLLMTLRLWSS

SEQ ID NO: 27 - protein, 283 aa, Artificial Sequence
  Radium-1 alpha chain with double Myc-tag and murinised constant region
MKRILGALLGLLSAQVCCVREQKLISEEDLEQKLISEEDLGIQVEQSPPDLILQEGANSTLRCNFSDSVNNLQWFHQNPWGQLINLFYIPSGTKQNGRLSATTVATERYSLLYISSSQTTDSGVYFCAVNAGNMLTFGGGTRLMVKPIQNPEPAVYQLKDPRSQDSTLCLFTDFDSQINVPKTMESGTFITDKTVLDMKAMDSKSNGAIAWSNQTSFTCQDIFKETNATYPSSDVPCDATLTEKSFETDMNLNFQNLSVMGLRILLLKVAGFNLLMTLRLWSS

SEQ ID NO: 28 - protein, 283 aa, Artificial Sequence
  Radium-1 alpha-chain with double Myc-tag and cysteine-modified murinised constant region
MKRILGALLGLLSAQVCCVREQKLISEEDLEQKLISEEDLGIQVEQSPPDLILQEGANSTLRCNFSDSVNNLQWFHQNPWGQLINLFYIPSGTKQNGRLSATTVATERYSLLYISSSQTTDSGVYFCAVNAGNMLTFGGGTRLMVKPIQNPEPAVYQLKDPRSQDSTLCLFTDFDSQINVPKTMESGTFITDKCVLDMKAMDSKSNGAIAWSNQTSFTCQDIFKETNATYPSSDVPCDATLTEKSFETDMNLNFQNLSVMGLRILLLKVAGFNLLMTLRLWSS

SEQ ID NO: 29 - protein, 125 aa, Mus musculus
EDLRNVTPPKVSLFEPSKAEIANKQKATLVCLARGFFPDHVELSWWVNGKEVHSGVSTDPQAYKESNYSYCLSSRLRVSATFWHNPRNHFRCQVQFHGLSEEDKWPEGSPKPVTQNISAEAWGRA

SEQ ID NO: 30 - protein, 125 aa, Artificial Sequence
  Cysteine-modified murinised Radium-1 beta-chain constant region
EDLRNVTPPKVSLFEPSKAEIANKQKATLVCLARGFFPDHVELSWWVNGKEVHSGVCTDPQAYKESNYSYCLSSRLRVSATFWHNPRNHFRCQVQFHGLSEEDKWPEGSPKPVTQNISAEAWGRA

SEQ ID NO: 31 - protein, 256 aa, Artificial Sequence
  Radium-1 beta-chain with murinised constant region
MGIRLLCRVAFCFLAVGLVDVKVTQSSRYLVKRTGEKVFLECVQDMDHENMFWYRQDPGLGLRLIYFSYDVKMKEKGDIPEGYSVSREKKERFSLILESASTNQTSMYLCASSSGVTGELFFGEGSRLTVLEDLRNVTPPKVSLFEPSKAEIANKQKATLVCLARGFFPDHVELSWWVNGKEVHSGVSTDPQAYKESNYSYCLSSRLRVSATFWHNPRNHFRCQVQFHGLSEEDKWPEGSPKPVTQNISAEAWGRA

SEQ ID NO: 32 - protein, 256 aa, Artificial Sequence
  Radium-1 beta-chain with cysteine-modified murinised constant region
MGIRLLCRVAFCFLAVGLVDVKVTQSSRYLVKRTGEKVFLECVQDMDHENMFWYRQDPGLGLRLIYFSYDVKMKEKGDIPEGYSVSREKKERFSLILESASTNQTSMYLCASSSGVTGELFFGEGSRLTVLEDLRNVTPPKVSLFEPSKAEIANKQKATLVCLARGFFPDHVELSWWVNGKEVHSGVCTDPQAYKESNYSYCLSSRLRVSATFWHNPRNHFRCQVQFHGLSEEDKWPEGSPKPVTQNISAEAWGRA

SEQ ID NO: 33 - protein, 604 aa, Artificial Sequence
  Radium-1 scTCR with 2A linker
MKRILGALLGLLSAQVCCVRGIQVEQSPPDLILQEGANSTLRCNFSDSVNNLQWFHQNPWGQLINLFYIPSGTKQNGRLSATTVATERYSLLYISSSQTTDSGVYFCAVNAGNMLTFGGGTRLMVKPHIQNPDPAVYQLRDSKSSDKSVCLFTDFDSQTNVSQSKDSDVYITDKTVLDMRSMDFKSNSAVAWSNKSDFACANAFNNSIIPEDTFFPSPESSCDVKLVEKSFETDTNLNFQNLSVIGFRILLLKVAGFNLLMTLRLWSSRAKRGSGATNFSLLKQAGDVEENPGPMGIRLLCRVAFCFLAVGLVDVKVTQSSRYLVKRTGEKVFLECVQDMDHENMFWYRQDPGLGLRLIYFSYDVKMKEKGDIPEGYSVSREKKERFSLILESASTNQTSMYLCASSSGVTGELFFGEGSRLTVLEDLKNVFPPEVAVFEPSEAEISHTQKATLVCLATGFYPDHVELSWWVNGKEVHSGVSTDPQPLKEQPALNDSRYCLSSRLRVSATFWQNPRNHFRCQVQFYGLSENDEWTQDRAKPVTQIVSAEAWGRADCGFTSESYQQGVLSATILYEILLGKATLYAVLVSALVLMAMVKRKDSRG

SEQ ID NO: 34 - protein, 604 aa, Artificial Sequence
  Cysteine-modified Radium-1 scTCR with 2A linker
MKRILGALLGLLSAQVCCVRGIQVEQSPPDLILQEGANSTLRCNFSDSVNNLQWFHQNPWGQLINLFYIPSGTKQNGRLSATTVATERYSLLYISSSQTTDSGVYFCAVNAGNMLTFGGGTRLMVKPHIQNPDPAVYQLRDSKSSDKSVCLFTDFDSQTNVSQSKDSDVYITDKCVLDMRSMDFKSNSAVAWSNKSDFACANAFNNSIIPEDTFFPSPESSCDVKLVEKSFETDTNLNFQNLSVIGFRILLLKVAGFNLLMTLRLWSSRAKRGSGATNFSLLKQAGDVEENPGPMGIRLLCRVAFCFLAVGLVDVKVTQSSRYLVKRTGEKVFLECVQDMDHENMFWYRQDPGLGLRLIYFSYDVKMKEKGDIPEGYSVSREKKERFSLILESASTNQTSMYLCASSSGVTGELFFGEGSRLTVLEDLKNVFPPEVAVFEPSEAEISHTQKATLVCLATGFYPDHVELSWWVNGKEVHSGVCTDPQPLKEQPALNDSRYCLSSRLRVSATFWQNPRNHFRCQVQFYGLSENDEWTQDRAKPVTQIVSAEAWGRADCGFTSESYQQGVLSATILYEILLGKATLYAVLVSALVLMAMVKRKDSRG

SEQ ID NO: 35 - protein, 624 aa, Artificial Sequence
  Double Myc-tagged Radium-1 scTCR with 2A linker
MKRILGALLGLLSAQVCCVREQKLISEEDLEQKLISEEDLGIQVEQSPPDLILQEGANSTLRCNFSDSVNNLQWFHQNPWGQLINLFYIPSGTKQNGRLSATTVATERYSLLYISSSQTTDSGVYFCAVNAGNMLTFGGGTRLMVKPHIQNPDPAVYQLRDSKSSDKSVCLFTDFDSQTNVSQSKDSDVYITDKTVLDMRSMDFKSNSAVAWSNKSDFACANAFNNSIIPEDTFFPSPESSCDVKLVEKSFETDTNLNFQNLSVIGFRILLLKVAGFNLLMTLRLWSSRAKRGSGATNFSLLKQAGDVEENPGPMGIRLLCRVAFCFLAVGLVDVKVTQSSRYLVKRTGEKVFLECVQDMDHENMFWYRQDPGLGLRLIYFSYDVKMKEKGDIPEGYSVSREKKERFSLILESASTNQTSMYLCASSSGVTGELFFGEGSRLTVLEDLKNVFPPEVAVFEPSEAEISHTQKATLVCLATGFYPDHVELSWWVNGKEVHSGVSTDPQPLKEQPALNDSRYCLSSRLRVSATFWQNPRNHFRCQVQFYGLSENDEWTQDRAKPVTQIVSAEAWGRADCGFTSESYQQGVLSATILYEILLGKATLYAVLVSALVLMAMVKRKDSRG

SEQ ID NO: 36 - protein, 624 aa, Artificial Sequence
  Double Myc-tagged cysteine-modified Radium-1 scTCR with 2A linker
MKRILGALLGLLSAQVCCVREQKLISEEDLEQKLISEEDLGIQVEQSPPDLILQEGANSTLRCNFSDSVNNLQWFHQNPWGQLINLFYIPSGTKQNGRLSATTVATERYSLLYISSSQTTDSGVYFCAVNAGNMLTFGGGTRLMVKPHIQNPDPAVYQLRDSKSSDKSVCLFTDFDSQTNVSQSKDSDVYITDKCVLDMRSMDFKSNSAVAWSNKSDFACANAFNNSIIPEDTFFPSPESSCDVKLVEKSFETDTNLNFQNLSVIGFRILLLKVAGFNLLMTLRLWSSRAKRGSGATNFSLLKQAGDVEENPGPMGIRLLCRVAFCFLAVGLVDVKVTQSSRYLVKRTGEKVFLECVQDMDHENMFWYRQDPGLGLRLIYFSYDVKMKEKGDIPEGYSVSREKKERFSLILESASTNQTSMYLCASSSGVTGELFFGEGSRLTVLEDLKNVFPPEVAVFEPSEAEISHTQKATLVCLATGFYPDHVELSWWVNGKEVHSGVCTDPQPLKEQPALNDSRYCLSSRLRVSATFWQNPRNHFRCQVQFYGLSENDEWTQDRAKPVTQIVSAEAWGRADCGFTSESYQQGVLSATILYEILLGKATLYAVLVSALVLMAMVKRKDSRG

SEQ ID NO: 37 - protein, 545 aa, Artificial Sequence
  Radium-1 scTCR with murinised constant regions and 2A linker
MKRILGALLGLLSAQVCCVRGIQVEQSPPDLILQEGANSTLRCNFSDSVNNLQWFHQNPWGQLINLFYIPSGTKQNGRLSATTVATERYSLLYISSSQTTDSGVYFCAVNAGNMLTFGGGTRLMVKPIQNPEPAVYQLKDPRSQDSTLCLFTDFDSQINVPKTMESGTFITDKTVLDMKAMDSKSNGAIAWSNQTSFTCQDIFKETNATYPSSDVPCDATLTEKSFETDMNLNFQNLSVMGLRILLLKVAGFNLLMTLRLWSSRAKRGSGATNFSLLKQAGDVEENPGPMGIRLLCRVAFCFLAVGLVDVKVTQSSRYLVKRTGEKVFLECVQDMDHENMFWYRQDPGLGLRLIYFSYDVKMKEKGDIPEGYSVSREKKERFSLILESASTNQTSMYLCASSSGVTGELFFGEGSRLTVLEDLRNVTPPKVSLFEPSKAEIANKQKATLVCLARGFFPDHVELSWWVNGKEVHSGVSTDPQAYKESNYSYCLSSRLRVSATFWHNPRNHFRCQVQFHGLSEEDKWPEGSPKPVTQNISAEAWGRA

SEQ ID NO: 38 - protein, 545 aa, Artificial Sequence
  Radium-1 scTCR with cysteine-modified murinised constant regions and 2A linker
MKRILGALLGLLSAQVCCVRGIQVEQSPPDLILQEGANSTLRCNFSDSVNNLQWFHQNPWGQLINLFYIPSGTKQNGRLSATTVATERYSLLYISSSQTTDSGVYFCAVNAGNMLTFGGGTRLMVKPIQNPEPAVYQLKDPRSQDSTLCLFTDFDSQINVPKTMESGTFITDKCVLDMKAMDSKSNGAIAWSNQTSFTCQDIFKETNATYPSSDVPCDATLTEKSFETDMNLNFQNLSVMGLRILLLKVAGFNLLMTLRLWSSRAKRGSGATNFSLLKQAGDVEENPGPMGIRLLCRVAFCFLAVGLVDVKVTQSSRYLVKRTGEKVFLECVQDMDHENMFWYRQDPGLGLRLIYFSYDVKMKEKGDIPEGYSVSREKKERFSLILESASTNQTSMYLCASSSGVTGELFFGEGSRLTVLEDLRNVTPPKVSLFEPSKAEIANKQKATLVCLARGFFPDHVELSWWVNGKEVHSGVCTDPQAYKESNYSYCLSSRLRVSATFWHNPRNHFRCQVQFHGLSEEDKWPEGSPKPVTQNISAEAWGRA

SEQ ID NO: 39 - protein, 565 aa, Artificial Sequence
  Double Myc-tagged Radium-1 scTCR with murinised constant regions
MKRILGALLGLLSAQVCCVREQKLISEEDLEQKLISEEDLGIQVEQSPPDLILQEGANSTLRCNFSDSVNNLQWFHQNPWGQLINLFYIPSGTKQNGRLSATTVATERYSLLYISSSQTTDSGVYFCAVNAGNMLTFGGGTRLMVKPIQNPEPAVYQLKDPRSQDSTLCLFTDFDSQINVPKTMESGTFITDKTVLDMKAMDSKSNGAIAWSNQTSFTCQDIFKETNATYPSSDVPCDATLTEKSFETDMNLNFQNLSVMGLRILLLKVAGFNLLMTLRLWSSRAKRGSGATNFSLLKQAGDVEENPGPMGIRLLCRVAFCFLAVGLVDVKVTQSSRYLVKRTGEKVFLECVQDMDHENMFWYRQDPGLGLRLIYFSYDVKMKEKGDIPEGYSVSREKKERFSLILESASTNQTSMYLCASSSGVTGELFFGEGSRLTVLEDLRNVTPPKVSLFEPSKAEIANKQKATLVCLARGFFPDHVELSWWVNGKEVHSGVSTDPQAYKESNYSYCLSSRLRVSATFWHNPRNHFRCQVQFHGLSEEDKWPEGSPKPVTQNISAEAWGRA

SEQ ID NO: 40 - protein, 565 aa, Artificial Sequence
  Double Myc-tagged Radium-1 scTCR with cysteine-modified murinised constant regions and 2A linker
MKRILGALLGLLSAQVCCVREQKLISEEDLEQKLISEEDLGIQVEQSPPDLILQEGANSTLRCNFSDSVNNLQWFHQNPWGQLINLFYIPSGTKQNGRLSATTVATERYSLLYISSSQTTDSGVYFCAVNAGNMLTFGGGTRLMVKPIQNPEPAVYQLKDPRSQDSTLCLFTDFDSQINVPKTMESGTFITDKCVLDMKAMDSKSNGAIAWSNQTSFTCQDIFKETNATYPSSDVPCDATLTEKSFETDMNLNFQNLSVMGLRILLLKVAGFNLLMTLRLWSSRAKRGSGATNFSLLKQAGDVEENPGPMGIRLLCRVAFCFLAVGLVDVKVTQSSRYLVKRTGEKVFLECVQDMDHENMFWYRQDPGLGLRLIYFSYDVKMKEKGDIPEGYSVSREKKERFSLILESASTNQTSMYLCASSSGVTGELFFGEGSRLTVLEDLRNVTPPKVSLFEPSKAEIANKQKATLVCLARGFFPDHVELSWWVNGKEVHSGVCTDPQAYKESNYSYCLSSRLRVSATFWHNPRNHFRCQVQFHGLSEEDKWPEGSPKPVTQNISAEAWGRA

SEQ ID NO: 41 - DNA, 1815 bp, Artificial Sequence
  Encodes SEQ ID NO: 33
atgaagaggatattgggagctctgctggggctcttgagtgcccaggtttgctgtgtgagaggaatacaagtggagcagagtcctccagacctgattctccaggagggagccaattccacgctgcggtgcaatttttctgactctgtgaacaatttgcagtggtttcatcaaaacccttggggacagctcatcaacctgttttacattccctcagggacaaaacagaatggaagattaagcgccacgactgtcgctacggaacgctacagcttattgtacatttcctcttcccagaccacagactcaggcgtttatttctgtgctgtgaatgcaggcaacatgctcacctttggagggggaacaaggttaatggtcaaaccccatatccagaaccctgaccctgccgtgtaccagctgagagactctaaatccagtgacaagtctgtctgcctattcaccgattttgattctcaaacaaatgtgtcacaaagtaaggattctgatgtgtatatcacagacaaaactgtgctagacatgaggtctatggacttcaagagcaacagtgctgtggcctggagcaacaaatctgactttgcatgtgcaaacgccttcaacaacagcattattccagaagacaccttcttccccagcccagaaagttcctgtgatgtcaagctggtcgagaaaagctttgaaacagatacgaacctaaactttcaaaacctgtcagtgattgggttccgaatcctcctcctaaaagtggccgggtttaatctgctcatgacgctgcggctgtggtccagcagagccaagagaggcagcggcgccaccaacttcagcctgctgaagcaggccggcgacgtggaagagaaccctggaccaatgggaatcaggctcctctgtcgtgtggccttttgtttcctggctgtaggcctcgtagatgtgaaagtaacccagagctcgagatatctagtcaaaaggacgggagagaaagtttttctggaatgtgtccaggatatggaccatgaaaatatgttctggtatcgacaagacccaggtctggggctacggctgatctatttctcatatgatgttaaaatgaaagaaaaaggagatattcctgaggggtacagtgtctctagagagaagaaggagcgcttctccctgattctggagtccgccagcaccaaccagacatctatgtacctctgtgccagcagttctggagtcaccggggagctgttttttggagaaggctctaggctgaccgtactggaggacctgaaaaacgtgttcccacccgaggtcgctgtgtttgagccatcagaagcagagatctcccacacccaaaaggccacactggtgtgcctggccacaggcttctaccccgaccacgtggagctgagctggtgggtgaatgggaaggaggtgcacagtggggtcagcacagacccgcagcccctcaaggagcagcccgccctcaatgactccagatactgcctgagcagccgcctgagggtctcggccaccttctggcagaacccccgcaaccacttccgctgtcaagtccagttctacgggctctcggagaatgacgagtggacccaggatagggccaaacctgtcacccagatcgtcagcgccgaggcctggggtagagcagactgtggcttcacctccgagtcttaccagcaaggggtcctgtctgccaccatcctctatgagatcttgctagggaaggccaccttgtatgccgtgctggtcagtgccctcgtgctgatggccatggtcaagagaaaggattccagaggctag

SEQ ID NO: 42 - DNA, 1815 bp, Artificial Sequence
  Encodes SEQ ID NO: 34
atgaagaggatattgggagctctgctggggctcttgagtgcccaggtttgctgtgtgagaggaatacaagtggagcagagtcctccagacctgattctccaggagggagccaattccacgctgcggtgcaatttttctgactctgtgaacaatttgcagtggtttcatcaaaacccttggggacagctcatcaacctgttttacattccctcagggacaaaacagaatggaagattaagcgccacgactgtcgctacggaacgctacagcttattgtacatttcctcttcccagaccacagactcaggcgtttatttctgtgctgtgaatgcaggcaacatgctcacctttggagggggaacaaggttaatggtcaaaccccatatccagaaccctgaccctgccgtgtaccagctgagagactctaaatccagtgacaagtctgtctgcctattcaccgattttgattctcaaacaaatgtgtcacaaagtaaggattctgatgtgtatatcacagacaaatgcgtgctagacatgaggtctatggacttcaagagcaacagtgctgtggcctggagcaacaaatctgactttgcatgtgcaaacgccttcaacaacagcattattccagaagacaccttcttccccagcccagaaagttcctgtgatgtcaagctggtcgagaaaagctttgaaacagatacgaacctaaactttcaaaacctgtcagtgattgggttccgaatcctcctcctaaaagtggccgggtttaatctgctcatgacgctgcggctgtggtccagcagagccaagagaggcagcggcgccaccaacttcagcctgctgaagcaggccggcgacgtggaagagaaccctggaccaatgggaatcaggctcctctgtcgtgtggccttttgtttcctggctgtaggcctcgtagatgtgaaagtaacccagagctcgagatatctagtcaaaaggacgggagagaaagtttttctggaatgtgtccaggatatggaccatgaaaatatgttctggtatcgacaagacccaggtctggggctacggctgatctatttctcatatgatgttaaaatgaaagaaaaaggagatattcctgaggggtacagtgtctctagagagaagaaggagcgcttctccctgattctggagtccgccagcaccaaccagacatctatgtacctctgtgccagcagttctggagtcaccggggagctgttttttggagaaggctctaggctgaccgtactggaggacctgaaaaacgtgttcccacccgaggtcgctgtgtttgagccatcagaagcagagatctcccacacccaaaaggccacactggtgtgcctggccacaggcttctaccccgaccacgtggagctgagctggtgggtgaatgggaaggaggtgcacagtggggtctgtacagacccgcagcccctcaaggagcagcccgccctcaatgactccagatactgcctgagcagccgcctgagggtctcggccaccttctggcagaacccccgcaaccacttccgctgtcaagtccagttctacgggctctcggagaatgacgagtggacccaggatagggccaaacctgtcacccagatcgtcagcgccgaggcctggggtagagcagactgtggcttcacctccgagtcttaccagcaaggggtcctgtctgccaccatcctctatgagatcttgctagggaaggccaccttgtatgccgtgctggtcagtgccctcgtgctgatggccatggtcaagagaaaggattccagaggctag

SEQ ID NO: 43 - DNA, 1875 bp, Artificial Sequence
  Encodes SEQ ID NO: 35
atgaagaggatattgggagctctgctggggctcttgagtgcccaggtttgctgtgtgagagagcagaagctgatcagcgaggaggacctggagcagaagctgatcagcgaggaggacctgggaatacaagtggagcagagtcctccagacctgattctccaggagggagccaattccacgctgcggtgcaatttttctgactctgtgaacaatttgcagtggtttcatcaaaacccttggggacagctcatcaacctgttttacattccctcagggacaaaacagaatggaagattaagcgccacgactgtcgctacggaacgctacagcttattgtacatttcctcttcccagaccacagactcaggcgtttatttctgtgctgtgaatgcaggcaacatgctcacctttggagggggaacaaggttaatggtcaaaccccatatccagaaccctgaccctgccgtgtaccagctgagagactctaaatccagtgacaagtctgtctgcctattcaccgattttgattctcaaacaaatgtgtcacaaagtaaggattctgatgtgtatatcacagacaaaactgtgctagacatgaggtctatggacttcaagagcaacagtgctgtggcctggagcaacaaatctgactttgcatgtgcaaacgccttcaacaacagcattattccagaagacaccttcttccccagcccagaaagttcctgtgatgtcaagctggtcgagaaaagctttgaaacagatacgaacctaaactttcaaaacctgtcagtgattgggttccgaatcctcctcctaaaagtggccgggtttaatctgctcatgacgctgcggctgtggtccagcagagccaagagaggcagcggcgccaccaacttcagcctgctgaagcaggccggcgacgtggaagagaaccctggaccaatgggaatcaggctcctctgtcgtgtggccttttgtttcctggctgtaggcctcgtagatgtgaaagtaacccagagctccagatatctagtcaaaaggacgggagagaaagtttttctggaatgtgtccaggatatggaccatgaaaatatgttctggtatcgacaagacccaggtctggggctacggctgatctatttctcatatgatgttaaaatgaaagaaaaaggagatattcctgaggggtacagtgtctctagagagaagaaggagcgcttctccctgattctggagtccgccagcaccaaccagacatctatgtacctctgtgccagcagttctggagtcaccggggagctgttttttggagaaggctctaggctgaccgtactggaggacctgaaaaacgtgttcccacccgaggtcgctgtgtttgagccatcagaagcagagatctcccacacccaaaaggccacactggtgtgcctggccacaggcttctaccccgaccacgtggagctgagctggtgggtgaatgggaaggaggtgcacagtggggtcagcacagacccgcagcccctcaaggagcagcccgccctcaatgactccagatactgcctgagcagccgcctgagggtctcggccaccttctggcagaacccccgcaaccacttccgctgtcaagtccagttctacgggctctcggagaatgacgagtggacccaggatagggccaaacctgtcacccagatcgtcagcgccgaggcctggggtagagcagactgtggcttcacctccgagtcttaccagcaaggggtcctgtctgccaccatcctctatgagatcttgctagggaaggccaccttgtatgccgtgctggtcagtgccctcgtgctgatggccatggtcaagagaaaggattccagaggctag

SEQ ID NO: 44 - DNA, 1875 bp, Artificial Sequence
  Encodes SEQ ID NO: 36
atgaagaggatattgggagctctgctggggctcttgagtgcccaggtttgctgtgtgagagagcagaagctgatcagcgaggaggacctggagcagaagctgatcagcgaggaggacctgggaatacaagtggagcagagtcctccagacctgattctccaggagggagccaattccacgctgcggtgcaatttttctgactctgtgaacaatttgcagtggtttcatcaaaacccttggggacagctcatcaacctgttttacattccctcagggacaaaacagaatggaagattaagcgccacgactgtcgctacggaacgctacagcttattgtacatttcctcttcccagaccacagactcaggcgtttatttctgtgctgtgaatgcaggcaacatgctcacctttggagggggaacaaggttaatggtcaaaccccatatccagaaccctgaccctgccgtgtaccagctgagagactctaaatccagtgacaagtctgtctgcctattcaccgattttgattctcaaacaaatgtgtcacaaagtaaggattctgatgtgtatatcacagacaaatgcgtgctagacatgaggtctatggacttcaagagcaacagtgctgtggcctggagcaacaaatctgactttgcatgtgcaaacgccttcaacaacagcattattccagaagacaccttcttccccagcccagaaagttcctgtgatgtcaagctggtcgagaaaagctttgaaacagatacgaacctaaactttcaaaacctgtcagtgattgggttccgaatcctcctcctaaaagtggccgggtttaatctgctcatgacgctgcggctgtggtccagcagagccaagagaggcagcggcgccaccaacttcagcctgctgaagcaggccggcgacgtggaagagaaccctggaccaatgggaatcaggctcctctgtcgtgtggccttttgtttcctggctgtaggcctcgtagatgtgaaagtaacccagagctcgagatatctagtcaaaaggacgggagagaaagtttttctggaatgtgtccaggatatggaccatgaaaatatgttctggtatcgacaagacccaggtctggggctacggctgatctatttctcatatgatgttaaaatgaaagaaaaaggagatattcctgaggggtacagtgtctctagagagaagaaggagcgcttctccctgattctggagtccgccagcaccaaccagacatctatgtacctctgtgccagcagttctggagtcaccggggagctgttttttggagaaggctctaggctgaccgtactggaggacctgaaaaacgtgttcccacccgaggtcgctgtgtttgagccatcagaagcagagatctcccacacccaaaaggccacactggtgtgcctggccacaggcttctaccccgaccacgtggagctgagctggtgggtgaatgggaaggaggtgcacagtggggtctgtacagacccgcagcccctcaaggagcagcccgccctcaatgactccagatactgcctgagcagccgcctgagggtctcggccaccttctggcagaacccccgcaaccacttccgctgtcaagtccagttctacgggctctcggagaatgacgagtggacccaggatagggccaaacctgtcacccagatcgtcagcgccgaggcctggggtagagcagactgtggcttcacctccgagtcttaccagcaaggggtcctgtctgccaccatcctctatgagatcttgctagggaaggccaccttgtatgccgtgctggtcagtgccctcgtgctgatggccatggtcaagagaaaggattccagaggctag

SEQ ID NO: 45 - DNA, 1638 bp, Artificial Sequence
  Encodes SEQ ID NO: 37
atgaagaggatattgggagctctgctggggctcttgagtgcccaggtttgctgtgtgagaggaatacaagtggagcagagtcctccagacctgattctccaggagggagccaattccacgctgcggtgcaatttttctgactctgtgaacaatttgcagtggtttcatcaaaacccttggggacagctcatcaacctgttttacattccctcagggacaaaacagaatggaagattaagcgccacgactgtcgctacggaacgctacagcttattgtacatttcctcttcccagaccacagactcaggcgtttatttctgtgctgtgaatgcaggcaacatgctcacctttggagggggaacaaggttaatggtcaaacccatccagaacccagaacctgctgtgtaccagttaaaagatcctcggtctcaggacagcaccctctgcctgttcaccgactttgactcccaaatcaatgtgccgaaaaccatggaatctggaacgttcatcactgacaaaactgtgctggacatgaaagctatggattccaagagcaatggggccattgcctggagcaaccagacaagcttcacctgccaagatatcttcaaagagaccaacgccacctaccccagttcagacgttccctgtgatgccacgttgactgagaaaagctttgaaacagatatgaacctaaactttcaaaacctgtcagttatgggactccgaatcctcctgctgaaagtagccggatttaacctgctcatgacgctgaggctgtggtccagtagagccaagagaggcagcggcgccaccaacttcagcctgctgaagcaggccggcgacgtggaagagaaccctggaccaatgggaatcaggctcctctgtcgtgtggccttttgtttcctggctgtaggcctcgtagatgtgaaagtaacccagagctcgagatatctagtcaaaaggacgggagagaaagtttttctggaatgtgtccaggatatggaccatgaaaatatgttctggtatcgacaagacccaggtctggggctacggctgatctatttctcatatgatgttaaaatgaaagaaaaaggagatattcctgaggggtacagtgtctctagagagaagaaggagcgcttctccctgattctggagtccgccagcaccaaccagacatctatgtacctctgtgccagcagttctggagtcaccggggagctgttttttggagaaggctctaggctgaccgtactggaggatctgagaaatgtgactccacccaaggtctccttgtttgagccatcaaaagcagagattgcaaacaaacaaaaggctaccctcgtgtgcttggccaggggcttcttccctgaccacgtggagctgagctggtgggtgaatggcaaggaggtccacagtggggtcagcacggaccctcaggcctacaaggagagcaattatagctactgcctgagcagccgcctgagggtctctgctaccttctggcacaatcctcgaaaccacttccgctgccaagtgcagttccatgggctttcagaggaggacaagtggccagagggctcacccaaacctgtcacacagaacatcagtgcagaggcctggggccgagcatag

SEQ ID NO: 46 - DNA, 1638 bp, Artificial Sequence
  Encodes SEQ ID NO: 38
atgaagaggatattgggagctctgctggggctcttgagtgcccaggtttgctgtgtgagaggaatacaagtggagcagagtcctccagacctgattctccaggagggagccaattccacgctgcggtgcaatttttctgactctgtgaacaatttgcagtggtttcatcaaaacccttggggacagctcatcaacctgttttacattccctcagggacaaaacagaatggaagattaagcgccacgactgtcgctacggaacgctacagcttattgtacatttcctcttcccagaccacagactcaggcgtttatttctgtgctgtgaatgcaggcaacatgctcacctttggagggggaacaaggttaatggtcaaacccatccagaacccagaacctgctgtgtaccagttaaaagatcctcggtctcaggacagcaccctctgcctgttcaccgactttgactcccaaatcaatgtgccgaaaaccatggaatctggaacgttcatcactgacaaatgcgtgctggacatgaaagctatggattccaagagcaatggggccattgcctggagcaaccagacaagcttcacctgccaagatatcttcaaagagaccaacgccacctaccccagttcagacgttccctgtgatgccacgttgactgagaaaagctttgaaacagatatgaacctaaactttcaaaacctgtcagttatgggactccgaatcctcctgctgaaagtagccggatttaacctgctcatgacgctgaggctgtggtccagtagagccaagagaggcagcggcgccaccaacttcagcctgctgaagcaggccggcgacgtggaagagaaccctggaccaatgggaatcaggctcctctgtcgtgtggccttttgtttcctggctgtaggcctcgtagatgtgaaagtaacccagagctcgagatatctagtcaaaaggacgggagagaaagtttttctggaatgtgtccaggatatggaccatgaaaatatgttctggtatcgacaagacccaggtctggggctacggctgatctatttctcatatgatgttaaaatgaaagaaaaaggagatattcctgaggggtacagtgtctctagagagaagaaggagcgcttctccctgattctggagtccgccagcaccaaccagacatctatgtacctctgtgccagcagttctggagtcaccggggagctgttttttggagaaggctctaggctgaccgtactggaggatctgagaaatgtgactccacccaaggtctccttgtttgagccatcaaaagcagagattgcaaacaaacaaaaggctaccctcgtgtgcttggccaggggcttcttccctgaccacgtggagctgagctggtgggtgaatggcaaggaggtccacagtggggtctgtacggaccctcaggcctacaaggagagcaattatagctactgcctgagcagccgcctgagggtctctgctaccttctggcacaatcctcgaaaccacttccgctgccaagtgcagttccatgggctttcagaggaggacaagtggccagagggctcacccaaacctgtcacacagaacatcagtgcagaggcctggggccgagcatag

SEQ ID NO: 47 - DNA, 1698 bp, Artificial Sequence
  Encodes SEQ ID NO: 39
atgaagaggatattgggagctctgctggggctcttgagtgcccaggtttgctgtgtgagagagcagaagctgatcagcgaggaggacctggagcagaagctgatcagcgaggaggacctgggaatacaagtggagcagagtcctccagacctgattctccaggagggagccaattccacgctgcggtgcaatttttctgactctgtgaacaatttgcagtggtttcatcaaaacccttggggacagctcatcaacctgttttacattccctcagggacaaaacagaatggaagattaagcgccacgactgtcgctacggaacgctacagcttattgtacatttcctcttcccagaccacagactcaggcgtttatttctgtgctgtgaatgcaggcaacatgctcacctttggagggggaacaaggttaatggtcaaacccatccagaacccagaacctgctgtgtaccagttaaaagatcctcggtctcaggacagcaccctctgcctgttcaccgactttgactcccaaatcaatgtgccgaaaaccatggaatctggaacgttcatcactgacaaaactgtgctggacatgaaagctatggattccaagagcaatggggccattgcctggagcaaccagacaagcttcacctgccaagatatcttcaaagagaccaacgccacctaccccagttcagacgttccctgtgatgccacgttgactgagaaaagctttgaaacagatatgaacctaaactttcaaaacctgtcagttatgggactccgaatcctcctgctgaaagtagccggatttaacctgctcatgacgctgaggctgtggtccagtagagccaagagaggcagcggcgccaccaacttcagcctgctgaagcaggccggcgacgtggaagagaaccctggaccaatgggaatcaggctcctctgtcgtgtggccttttgtttcctggctgtaggcctcgtagatgtgaaagtaacccagagctcgagatatctagtcaaaaggacgggagagaaagtttttctggaatgtgtccaggatatggaccatgaaaatatgttctggtatcgacaagacccaggtctggggctacggctgatctatttctcatatgatgttaaaatgaaagaaaaaggagatattcctgaggggtacagtgtctctagagagaagaaggagcgcttctccctgattctggagtccgccagcaccaaccagacatctatgtacctctgtgccagcagttctggagtcaccggggagctgttttttggagaaggctctaggctgaccgtactggaggatctgagaaatgtgactccacccaaggtctccttgtttgagccatcaaaagcagagattgcaaacaaacaaaaggctaccctcgtgtgcttggccaggggcttcttccctgaccacgtggagctgagctggtgggtgaatggcaaggaggtccacagtggggtcagcacggaccctcaggcctacaaggagagcaattatagctactgcctgagcagccgcctgagggtctctgctaccttctggcacaatcctcgaaaccacttccgctgccaagtgcagttccatgggctttcagaggaggacaagtggccagagggctcacccaaacctgtcacacagaacatcagtgcagaggcctggggccgagcatag

SEQ ID NO: 48 - DNA, 1698 bp, Artificial Sequence
  Encodes SEQ ID NO: 40
atgaagaggatattgggagctctgctggggctcttgagtgcccaggtttgctgtgtgagagagcagaagctgatcagcgaggaggacctggagcagaagctgatcagcgaggaggacctgggaatacaagtggagcagagtcctccagacctgattctccaggagggagccaattccacgctgcggtgcaatttttctgactctgtgaacaatttgcagtggtttcatcaaaacccttggggacagctcatcaacctgttttacattccctcagggacaaaacagaatggaagattaagcgccacgactgtcgctacggaacgctacagcttattgtacatttcctcttcccagaccacagactcaggcgtttatttctgtgctgtgaatgcaggcaacatgctcacctttggagggggaacaaggttaatggtcaaacccatccagaacccagaacctgctgtgtaccagttaaaagatcctcggtctcaggacagcaccctctgcctgttcaccgactttgactcccaaatcaatgtgccgaaaaccatggaatctggaacgttcatcactgacaaatgcgtgctggacatgaaagctatggattccaagagcaatggggccattgcctggagcaaccagacaagcttcacctgccaagatatcttcaaagagaccaacgccacctaccccagttcagacgttccctgtgatgccacgttgactgagaaaagctttgaaacagatatgaacctaaactttcaaaacctgtcagttatgggactccgaatcctcctgctgaaagtagccggatttaacctgctcatgacgctgaggctgtggtccagtagagccaagagaggcagcggcgccaccaacttcagcctgctgaagcaggccggcgacgtggaagagaaccctggaccaatgggaatcaggctcctctgtcgtgtggccttttgtttcctggctgtaggcctcgtagatgtgaaagtaacccagagctcgagatatctagtcaaaaggacgggagagaaagtttttctggaatgtgtccaggatatggaccatgaaaatatgttctggtatcgacaagacccaggtctggggctacggctgatctatttctcatatgatgttaaaatgaaagaaaaaggagatattcctgaggggtacagtgtctctagagagaagaaggagcgcttctccctgattctggagtccgccagcaccaaccagacatctatgtacctctgtgccagcagttctggagtcaccggggagctgttttttggagaaggctctaggctgaccgtactggaggatctgagaaatgtgactccacccaaggtctccttgtttgagccatcaaaagcagagattgcaaacaaacaaaaggctaccctcgtgtgcttggccaggggcttcttccctgaccacgtggagctgagctggtgggtgaatggcaaggaggtccacagtggggtctgtacggaccctcaggcctacaaggagagcaattatagctactgcctgagcagccgcctgagggtctctgctaccttctggcacaatcctcgaaaccacttccgctgccaagtgcagttccatgggctttcagaggaggacaagtggccagagggctcacccaaacctgtcacacagaacatcagtgcagaggcctggggccgagcatag

SEQ ID NO: 49 - protein, 23 aa, Homo sapiens
SLVRLSSCVPVALMSAMTTSSSQ

SEQ ID NO: 50 - protein, 20 aa, Homo sapiens
MKRILGALLGLLSAQVCCVR

SEQ ID NO: 51 - protein, 16 aa, Homo sapiens
MGIRLLCRVAFCFLAV

SEQ ID NO: 52 - protein, 8 aa, picornavirus
  X (2)..(2): Val or Ile
  X (4)..(4): Any amino acid
DXEXNPGP

SEQ ID NO: 53 - DNA, 6 bp, Homo sapiens
aataaa

SEQ ID NO: 54 - protein, 9 aa, Homo sapiens
ILAKFLHWL

SEQ ID NO: 55 - protein, 19 aa, Homo sapiens
KSLVRLSSCVPVALMSAMT

SEQ ID NO: 56 - protein, 10 aa, Homo sapiens
EAAGIGILTV

SEQ ID NO: 57 - DNA, 35 bp, Artificial Sequence
  Site-directed mutagenesis forward primer
gaggaccagacccagaaggcggagctcgtggagac

SEQ ID NO: 58 - DNA, 35 bp, Artificial Sequence
  Site-directed mutagenesis reverse primer
gtctccacgagctccgccttctgggtctggtcctc

SEQ ID NO: 59 - protein, 15 aa, Escherichia coli
GGLNDIFEAQKIEWH

SEQ ID NO: 60 - protein, 95 aa, Homo sapiens
HIQNPDPAVYQLRDSKSSDKSVCLFTDFDSQTNVSQSKDSDVYITDKTVLDMRSMDFKSNSAVAWSNKSDFACANAFNNSIIPEDTFFPSPESSC

SEQ ID NO: 61 - protein, 95 aa, Artificial Sequence
  Cysteine-modified truncated Radium-1 alpha-chain constant region
HIQNPDPAVYQLRDSKSSDKSVCLFTDFDSQTNVSQSKDSDVYITDKCVLDMRSMDFKSNSAVAWSNKSDFACANAFNNSIIPEDTFFPSPESSC

SEQ ID NO: 62 - protein, 131 aa, Homo sapiens
EDLKNVFPPEVAVFEPSEAEISHTQKATLVCLATGFYPDHVELSWWVNGKEVHSGVSTDPQPLKEQPALNDSRYCLSSRLRVSATFWQNPRNHFRCQVQFYGLSENDEWTQDRAKPVTQIVSAEAWGRADC

SEQ ID NO: 63 - protein, 131 aa, Artificial Sequence
  Cysteine-modified truncated Radium-1 beta-chain constant region
EDLKNVFPPEVAVFEPSEAEISHTQKATLVCLATGFYPDHVELSWWVNGKEVHSGVCTDPQPLKEQPALNDSRYCLSSRLRVSATFWQNPRNHFRCQVQFYGLSENDEWTQDRAKPVTQIVSAEAWGRADC

SEQ ID NO: 64 - protein, 222 aa, Homo sapiens
MKRILGALLGLLSAQVCCVRGIQVEQSPPDLILQEGANSTLRCNFSDSVNNLQWFHQNPWGQLINLFYIPSGTKQNGRLSATTVATERYSLLYISSSQTTDSGVYFCAVNAGNMLTFGGGTRLMVKPHIQNPDPAVYQLRDSKSSDKSVCLFTDFDSQTNVSQSKDSDVYITDKTVLDMRSMDFKSNSAVAWSNKSDFACANAFNNSIIPEDTFFPSPESSC

SEQ ID NO: 65 - protein, 222 aa, Artificial Sequence
  Cysteine-modified truncated Radium-1 alpha-chain
MKRILGALLGLLSAQVCCVRGIQVEQSPPDLILQEGANSTLRCNFSDSVNNLQWFHQNPWGQLINLFYIPSGTKQNGRLSATTVATERYSLLYISSSQTTDSGVYFCAVNAGNMLTFGGGTRLMVKPHIQNPDPAVYQLRDSKSSDKSVCLFTDFDSQTNVSQSKDSDVYITDKCVLDMRSMDFKSNSAVAWSNKSDFACANAFNNSIIPEDTFFPSPESSC

SEQ ID NO: 66 - protein, 262 aa, Homo sapiens
MGIRLLCRVAFCFLAVGLVDVKVTQSSRYLVKRTGEKVFLECVQDMDHENMFWYRQDPGLGLRLIYFSYDVKMKEKGDIPEGYSVSREKKERFSLILESASTNQTSMYLCASSSGVTGELFFGEGSRLTVLEDLKNVFPPEVAVFEPSEAEISHTQKATLVCLATGFYPDHVELSWWVNGKEVHSGVSTDPQPLKEQPALNDSRYCLSSRLRVSATFWQNPRNHFRCQVQFYGLSENDEWTQDRAKPVTQIVSAEAWGRADC

SEQ ID NO: 67 - protein, 262 aa, Artificial Sequence
  Cysteine-modified truncated Radium-1 beta-chain
MGIRLLCRVAFCFLAVGLVDVKVTQSSRYLVKRTGEKVFLECVQDMDHENMFWYRQDPGLGLRLIYFSYDVKMKEKGDIPEGYSVSREKKERFSLILESASTNQTSMYLCASSSGVTGELFFGEGSRLTVLEDLKNVFPPEVAVFEPSEAEISHTQKATLVCLATGFYPDHVELSWWVNGKEVHSGVCTDPQPLKEQPALNDSRYCLSSRLRVSATFWQNPRNHFRCQVQFYGLSENDEWTQDRAKPVTQIVSAEAWGRADC

SEQ ID NO: 68 - protein, 510 aa, Artificial Sequence
  Soluble cysteine-modified Radium-1 scTCR with 2A linker
MKRILGALLGLLSAQVCCVRGIQVEQSPPDLILQEGANSTLRCNFSDSVNNLQWFHQNPWGQLINLFYIPSGTKQNGRLSATTVATERYSLLYISSSQTTDSGVYFCAVNAGNMLTFGGGTRLMVKPHIQNPDPAVYQLRDSKSSDKSVCLFTDFDSQTNVSQSKDSDVYITDKCVLDMRSMDFKSNSAVAWSNKSDFACANAFNNSIIPEDTFFPSPESSCRAKRGSGATNFSLLKQAGDVEENPGPMGIRLLCRVAFCFLAVGLVDVKVTQSSRYLVKRTGEKVFLECVQDMDHENMFWYRQDPGLGLRLIYFSYDVKMKEKGDIPEGYSVSREKKERFSLILESASTNQTSMYLCASSSGVTGELFFGEGSRLTVLEDLKNVFPPEVAVFEPSEAEISHTQKATLVCLATGFYPDHVELSWWVNGKEVHSGVCTDPQPLKEQPALNDSRYCLSSRLRVSATFWQNPRNHFRCQVQFYGLSENDEWTQDRAKPVTQIVSAEAWGRADC

SEQ ID NO: 69 - protein, 519 aa, Artificial Sequence
  Soluble cysteine-modified Radium-1 scTCR with C-terminal His-tag and linker
MKRILGALLGLLSAQVCCVRGIQVEQSPPDLILQEGANSTLRCNFSDSVNNLQWFHQNPWGQLINLFYIPSGTKQNGRLSATTVATERYSLLYISSSQTTDSGVYFCAVNAGNMLTFGGGTRLMVKPHIQNPDPAVYQLRDSKSSDKSVCLFTDFDSQTNVSQSKDSDVYITDKCVLDMRSMDFKSNSAVAWSNKSDFACANAFNNSIIPEDTFFPSPESSCRAKRGSGATNFSLLKQAGDVEENPGPMGIRLLCRVAFCFLAVGLVDVKVTQSSRYLVKRTGEKVFLECVQDMDHENMFWYRQDPGLGLRLIYFSYDVKMKEKGDIPEGYSVSREKKERFSLILESASTNQTSMYLCASSSGVTGELFFGEGSRLTVLEDLKNVFPPEVAVFEPSEAEISHTQKATLVCLATGFYPDHVELSWWVNGKEVHSGVCTDPQPLKEQPALNDSRYCLSSRLRVSATFWQNPRNHFRCQVQFYGLSENDEWTQDRAKPVTQIVSAEAWGRADCGGGHHHHHH

SEQ ID NO: 70 - DNA, 1530 bp, Artificial Sequence
  Encodes SEQ ID NO: 69
atgaagaggatattgggagctctgctggggctcttgagtgcccaggtttgctgtgtgagaggaatacaagtggagcagagtcctccagacctgattctccaggagggagccaattccacgctgcggtgcaatttttctgactctgtgaacaatttgcagtggtttcatcaaaacccttggggacagctcatcaacctgttttacattccctcagggacaaaacagaatggaagattaagcgccacgactgtcgctacggaacgctacagcttattgtacatttcctcttcccagaccacagactcaggcgtttatttctgtgctgtgaatgcaggcaacatgctcacctttggagggggaacaaggttaatggtcaaaccccatatccagaaccctgaccctgccgtgtaccagctgagagactctaaatccagtgacaagtctgtctgcctattcaccgattttgattctcaaacaaatgtgtcacaaagtaaggattctgatgtgtatatcacagacaaatgcgtgctagacatgaggtctatggacttcaagagcaacagtgctgtggcctggagcaacaaatctgactttgcatgtgcaaacgccttcaacaacagcattattccagaagacaccttcttccccagcccagaaagttcctgtagagccaagagaggcagcggcgccaccaacttcagcctgctgaagcaggccggcgacgtggaagagaaccctggaccaatgggaatcaggctcctctgtcgtgtggccttttgtttcctggctgtaggcctcgtagatgtgaaagtaacccagagctcgagatatctagtcaaaaggacgggagagaaagtttttctggaatgtgtccaggatatggaccatgaaaatatgttctggtatcgacaagacccaggtctggggctacggctgatctatttctcatatgatgttaaaatgaaagaaaaaggagatattcctgaggggtacagtgtctctagagagaagaaggagcgcttctccctgattctggagtccgccagcaccaaccagacatctatgtacctctgtgccagcagttctggagtcaccggggagctgttttttggagaaggctctaggctgaccgtactggaggacctgaaaaacgtgttcccacccgaggtcgctgtgtttgagccatcagaagcagagatctcccacacccaaaaggccacactggtgtgcctggccacaggcttctaccccgaccacgtggagctgagctggtgggtgaatgggaaggaggtgcacagtggggtctgtacagacccgcagcccctcaaggagcagcccgccctcaatgactccagatactgcctgagcagccgcctgagggtctcggccaccttctggcagaacccccgcaaccacttccgctgtcaagtccagttctacgggctctcggagaatgacgagtggacccaggatagggccaaacctgtcacccagatcgtcagcgccgaggcctggggtagagcagactgt

SEQ ID NO: 71 - DNA, 1557 bp, Artificial Sequence
  Encodes SEQ ID NO: 69
atgaagaggatattgggagctctgctggggctcttgagtgcccaggtttgctgtgtgagaggaatacaagtggagcagagtcctccagacctgattctccaggagggagccaattccacgctgcggtgcaatttttctgactctgtgaacaatttgcagtggtttcatcaaaacccttggggacagctcatcaacctgttttacattccctcagggacaaaacagaatggaagattaagcgccacgactgtcgctacggaacgctacagcttattgtacatttcctcttcccagaccacagactcaggcgtttatttctgtgctgtgaatgcaggcaacatgctcacctttggagggggaacaaggttaatggtcaaaccccatatccagaaccctgaccctgccgtgtaccagctgagagactctaaatccagtgacaagtctgtctgcctattcaccgattttgattctcaaacaaatgtgtcacaaagtaaggattctgatgtgtatatcacagacaaatgcgtgctagacatgaggtctatggacttcaagagcaacagtgctgtggcctggagcaacaaatctgactttgcatgtgcaaacgccttcaacaacagcattattccagaagacaccttcttccccagcccagaaagttcctgtagagccaagagaggcagcggcgccaccaacttcagcctgctgaagcaggccggcgacgtggaagagaaccctggaccaatgggaatcaggctcctctgtcgtgtggccttttgtttcctggctgtaggcctcgtagatgtgaaagtaacccagagctcgagatatctagtcaaaaggacgggagagaaagtttttctggaatgtgtccaggatatggaccatgaaaatatgttctggtatcgacaagacccaggtctggggctacggctgatctatttctcatatgatgttaaaatgaaagaaaaaggagatattcctgaggggtacagtgtctctagagagaagaaggagcgcttctccctgattctggagtccgccagcaccaaccagacatctatgtacctctgtgccagcagttctggagtcaccggggagctgttttttggagaaggctctaggctgaccgtactggaggacctgaaaaacgtgttcccacccgaggtcgctgtgtttgagccatcagaagcagagatctcccacacccaaaaggccacactggtgtgcctggccacaggcttctaccccgaccacgtggagctgagctggtgggtgaatgggaaggaggtgcacagtggggtctgtacagacccgcagcccctcaaggagcagcccgccctcaatgactccagatactgcctgagcagccgcctgagggtctcggccaccttctggcagaacccccgcaaccacttccgctgtcaagtccagttctacgggctctcggagaatgacgagtggacccaggatagggccaaacctgtcacccagatcgtcagcgccgaggcctggggtagagcagactgtggtggcggtcatcaccatcaccatcac

SEQ ID NO: 72 - protein, 107 aa, Homo sapiens
GIQVEQSPPDLILQEGANSTLRCNFSDSVNNLQWFHQNPWGQLINLFYIPSGTKQNGRLSATTVATERYSLLYISSSQTTDSGVYFCAVNAGNMLTFGGGTRLMVKP

SEQ ID NO: 73 - protein, 202 aa, Homo sapiens
GIQVEQSPPDLILQEGANSTLRCNFSDSVNNLQWFHQNPWGQLINLFYIPSGTKQNGRLSATTVATERYSLLYISSSQTTDSGVYFCAVNAGNMLTFGGGTRLMVKPHIQNPDPAVYQLRDSKSSDKSVCLFTDFDSQTNVSQSKDSDVYITDKTVLDMRSMDFKSNSAVAWSNKSDFACANAFNNSIIPEDTFFPSPESSC

SEQ ID NO: 74 - protein, 202 aa, Artificial Sequence
  Mature truncated cysteine-modified Radium-1 alpha-chain
GIQVEQSPPDLILQEGANSTLRCNFSDSVNNLQWFHQNPWGQLINLFYIPSGTKQNGRLSATTVATERYSLLYISSSQTTDSGVYFCAVNAGNMLTFGGGTRLMVKPHIQNPDPAVYQLRDSKSSDKSVCLFTDFDSQTNVSQSKDSDVYITDKCVLDMRSMDFKSNSAVAWSNKSDFACANAFNNSIIPEDTFFPSPESSC

SEQ ID NO: 75 - protein, 115 aa, Homo sapiens
GLVDVKVTQSSRYLVKRTGEKVFLECVQDMDHENMFWYRQDPGLGLRLIYFSYDVKMKEKGDIPEGYSVSREKKERFSLILESASTNQTSMYLCASSSGVTGELFFGEGSRLTVL

SEQ ID NO: 76 - protein, 246 aa, Homo sapiens
GLVDVKVTQSSRYLVKRTGEKVFLECVQDMDHENMFWYRQDPGLGLRLIYFSYDVKMKEKGDIPEGYSVSREKKERFSLILESASTNQTSMYLCASSSGVTGELFFGEGSRLTVLEDLKNVFPPEVAVFEPSEAEISHTQKATLVCLATGFYPDHVELSWWVNGKEVHSGVSTDPQPLKEQPALNDSRYCLSSRLRVSATFWQNPRNHFRCQVQFYGLSENDEWTQDRAKPVTQIVSAEAWGRADC

SEQ ID NO: 77 - protein, 246 aa, Artificial Sequence
  Mature truncated cysteine-modified Radium-1 beta-chain
GLVDVKVTQSSRYLVKRTGEKVFLECVQDMDHENMFWYRQDPGLGLRLIYFSYDVKMKEKGDIPEGYSVSREKKERFSLILESASTNQTSMYLCASSSGVTGELFFGEGSRLTVLEDLKNVFPPEVAVFEPSEAEISHTQKATLVCLATGFYPDHVELSWWVNGKEVHSGVCTDPQPLKEQPALNDSRYCLSSRLRVSATFWQNPRNHFRCQVQFYGLSENDEWTQDRAKPVTQIVSAEAWGRADC

SEQ ID NO: 78 - protein, 211 aa, Artificial Sequence
  Mature truncated cysteine-modified Radium-1 alpha-chain with linker and His-tag
GIQVEQSPPDLILQEGANSTLRCNFSDSVNNLQWFHQNPWGQLINLFYIPSGTKQNGRLSATTVATERYSLLYISSSQTTDSGVYFCAVNAGNMLTFGGGTRLMVKPHIQNPDPAVYQLRDSKSSDKSVCLFTDFDSQTNVSQSKDSDVYITDKCVLDMRSMDFKSNSAVAWSNKSDFACANAFNNSIIPEDTFFPSPESSCGGGHHHHHH

SEQ ID NO: 79 - protein, 255 aa, Artificial Sequence
  Mature truncated cysteine-modified Radium-1 beta-chain with linker and His-tag
GLVDVKVTQSSRYLVKRTGEKVFLECVQDMDHENMFWYRQDPGLGLRLIYFSYDVKMKEKGDIPEGYSVSREKKERFSLILESASTNQTSMYLCASSSGVTGELFFGEGSRLTVLEDLKNVFPPEVAVFEPSEAEISHTQKATLVCLATGFYPDHVELSWWVNGKEVHSGVCTDPQPLKEQPALNDSRYCLSSRLRVSATFWQNPRNHFRCQVQFYGLSENDEWTQDRAKPVTQIVSAEAWGRADCGGGHHHHHH

SEQ ID NO: 80 - protein, 10 aa, Artificial Sequence
  MART-1 26-35 peptide analogue
ELAGIGILTV

SEQ ID NO: 81 - protein, 227 aa, Artificial Sequence
  Mature truncated Radium-1 alpha-chain with 2A peptide-derived residues at C-terminus
GIQVEQSPPDLILQEGANSTLRCNFSDSVNNLQWFHQNPWGQLINLFYIPSGTKQNGRLSATTVATERYSLLYISSSQTTDSGVYFCAVNAGNMLTFGGGTRLMVKPHIQNPDPAVYQLRDSKSSDKSVCLFTDFDSQTNVSQSKDSDVYITDKTVLDMRSMDFKSNSAVAWSNKSDFACANAFNNSIIPEDTFFPSPESSCRAKRGSGATNFSLLKQAGDVEENPG

SEQ ID NO: 82 - protein, 227 aa, Artificial Sequence
  Mature truncated cysteine-modified Radium-1 alpha-chain with 2A peptide-derived residues at C-terminus
GIQVEQSPPDLILQEGANSTLRCNFSDSVNNLQWFHQNPWGQLINLFYIPSGTKQNGRLSATTVATERYSLLYISSSQTTDSGVYFCAVNAGNMLTFGGGTRLMVKPHIQNPDPAVYQLRDSKSSDKSVCLFTDFDSQTNVSQSKDSDVYITDKCVLDMRSMDFKSNSAVAWSNKSDFACANAFNNSIIPEDTFFPSPESSCRAKRGSGATNFSLLKQAGDVEENPG